European Patent Application EP 4 293 034 A1, published December 20, 2023. Title: A novel acylated derivate of phloretin and its use as antioxidant. Applicant: Consejo Superior de Investigaciones Cientificas (CSIC) ASOCIACIÓN CENTRO DE INVESTIGACIÓN COOPERATIVA EN BIOCIENCIAS - CICBIOGUNE GHENT UNIVERSITY. The sequence listing filed with the application follows.

SEQUENCE LISTING (2 sequences)

SEQ ID NO: 1 - protein, 488 aa, Thermoanaerobacterium thermosaccharolyticum
MALKNKVQLITYPDSLGGNLKTLNDVLEKYFSDVFGGVHILPPFPSSGDRGFAPITVSEIEPKFGTWYDIKKMAENFDILLDLMVNHVSRRSIYFQDFLKKGRKSEYADMFITLDKLWKDGKPVKGDIEKMFLRRTLPYSTFKIEETGEEEKVWTIFGKTDPSEQIDLDVNSHLVREFLLEVFKTFSNFGVKIVRLDAVGYVIKKIGTSCFFVEPEIVEFLDWAKGQAASYGIELLLEVHSQFEVQYKLAERGFLIYDFILPFTVLYTLINKSNEMLYHYLKNRPINQFTMLDCHDGIPVKPDLDGLIDTKKAKEVVDICVQRGANLSLIVGDKVKSEDGFDVHQINCTYVSALNCDDDAYLAARAIQFFTPGIPQVYYVGLLAGVNDFEAVKKTKEGREINRHNYGLKEIEESVQKNVVQRLLKLIRFRNEYEAFNGEFFIEDCRKDEIRLTWKKDDKRCSLFIDLKTYKTIIDYINENGEEVKYLV

SEQ ID NO: 2 - protein, 488 aa, Artificial Sequence
  Mutant of the sucrose 6'-phosphate phosphorylase from T. thermosaccharolyticum (TtSPP_R134A)
MALKNKVQLITYPDSLGGNLKTLNDVLEKYFSDVFGGVHILPPFPSSGDRGFAPITVSEIEPKFGTWYDIKKMAENFDILLDLMVNHVSRRSIYFQDFLKKGRKSEYADMFITLDKLWKDGKPVKGDIEKMFLARTLPYSTFKIEETGEEEKVWTIFGKTDPSEQIDLDVNSHLVREFLLEVFKTFSNFGVKIVRLDAVGYVIKKIGTSCFFVEPEIVEFLDWAKGQAASYGIELLLEVHSQFEVQYKLAERGFLIYDFILPFTVLYTLINKSNEMLYHYLKNRPINQFTMLDCHDGIPVKPDLDGLIDTKKAKEVVDICVQRGANLSLIVGDKVKSEDGFDVHQINCTYVSALNCDDDAYLAARAIQFFTPGIPQVYYVGLLAGVNDFEAVKKTKEGREINRHNYGLKEIEESVQKNVVQRLLKLIRFRNEYEAFNGEFFIEDCRKDEIRLTWKKDDKRCSLFIDLKTYKTIIDYINENGEEVKYLV